European Patent Application EP 4 116 410 A1, published January 11, 2023. Title: RECOMBINANT BCG, PREPARATION METHOD THEREFOR AND APPLICATION THEREOF. Applicant: Xuzhou Hairun Biotechnology Co., Ltd. Application EP20934400.1. The sequence listing filed with the application follows.

SEQUENCE LISTING (3 sequences)

SEQ ID NO: 1 - DNA, 62 bp, Artificial Sequence
  19ss Signal peptide
tatgaagcgtggactgacggtcgcggtagccggagccgccattctggtcgcaggtctttccg

SEQ ID NO: 2 - DNA, 53 bp, Artificial Sequence
  Primer F
ctggtgccgcgcggcagccatatgatgaaacgagttattaccctgtttgctgt

SEQ ID NO: 3 - DNA, 55 bp, Artificial Sequence
  Primer R
agtggtggtggtggtggtgctcgagaaactggaaatcatcgctgttatagttgtt